European Patent Specification EP 2 714 901 B1, published September 18, 2024. Title: Pest resistant plants. Applicant: Keygene N.V. The sequence listing filed with the application follows.

SEQUENCE LISTING (8 sequences)

SEQ ID NO: 1 - protein, 741 aa, Solanum habrochaites
CSHSTPSSMNGFEDARDRIRESFGKVELSPSSYDTAWVAMVPSKHSLNEPCFPQCLDWIIENQREDGSWGLNPSHPLLLKDSLSSTLACLLALTKWRVGDEQIKRGLGFIETQSWAIDNKDQISPLGFEIIFPSMIKSAEKLNLNLAINKRDSTIKRALQNEFTRNIEYMSEGFGELCDWKEIIKLHQRQNGSLFDSPATTAAALIYHQHDKKCYEYLNSILQQHKNWVPTMYPTKIHSLLCLVDTLQNLGVHRHFKSEIKKALDEIYRLWQQKNEEIFSNVTHCAMAFRLLRISYYDVSSDELAEFVDEEHFFATSGKYTSHVEILELHKASQLAIDHEKDDILDKINNWTRTFMEQKLLNNGFIDRMSKKEVELALRNFYIISDLAENRRYIKSYEENNFKILKAAYRSPNINNKDLFIFSIRDFELCQAQHQEELQQLKRWFEDCRLDQLGLSEQFISASYLCAIPIVPGPELSDARLVYAKYVMLLTIVDDHFESFASTDECLNIIELVERWDDYASVGYKSERVKVLFSMFYKSIEEIATIAEIKQGRSVKNHLINLWLKVMKLMLMERVEWCSGKTIPRIEEYLYVSSITFGSRLIPLTTQYFIGIKISKDLLESDEIYGLCNFTGIVLRLLNDLQDSKREQKEGSINLVTLLMKSISEEEAIMKMKEILEMKRRELFKMVLVQKKGSQLPQLCKEIFWRTCKWAHFTYSQTDRYRFPEEMENHIDEVFYKPLNH

SEQ ID NO: 2 - DNA, 2226 bp, Solanum habrochaites
tgcagccacagtaccccttcatcaatgaatggtttcgaagatgcaagggatagaataagggaaagttttgggaaagtagagttatctccttcttcctatgacacagcatgggtagctatggtcccttcaaaacattcactaaatgagccatgttttccacaatgtttggattggattattgaaaatcaaagagaagatggatcttggggactaaaccctagccatccattgcttcttaaggactcactttcttccactcttgcatgtttgcttgcactaaccaaatggagagttggagatgagcaaatcaaaagaggccttggctttattgaaacccagagttgggcaattgataacaaggatcaaatttcacctctaggatttgaaattatatttcccagtatgatcaagtctgcagaaaaactaaacttaaatctagcaattaacaaaagagattcaacaattaaaagagcattacagaatgagttcacgaggaatattgaatatatgagtgaaggatttggtgaattatgtgattggaaggaaataataaagttacatcaaaggcaaaatggttcattatttgattcaccagccactactgcagctgccttgatttaccatcagcatgataaaaaatgctatgaatatcttaattcaatcttgcaacaacacaaaaattgggttcccactatgtatccaacaaagatacattcattgctttgcttggttgatacacttcaaaatcttggagtacatcggcattttaaatcagaaataaagaaagccctagatgaaatatacaggctatggcaacaaaagaatgaagaaattttctcaaatgtcacccattgtgctatggcttttcgacttctaaggataagctactatgatgtctcctcagatgaactagcagaatttgtggatgaagaacatttctttgcaacaagtgggaaatatacaagtcatgttgaaattcttgaactccacaaagcatcacaattggctattgatcatgagaaagatgacattttggataagattaacaattggacaagaacatttatggagcaaaaactcttaaacaatggcttcatagataggatgtcaaaaaaggaggtggaacttgctttgaggaatttttatatcatatctgatctagcagaaaatagaagatatataaagtcatacgaagagaacaattttaaaatcttaaaagcagcttataggtcacctaacattaacaataaggacttgtttatattttcaatacgcgactttgaattatgccaagctcaacaccaagaagaacttcaacaactcaagaggtggtttgaagattgtagattggaccaactcggactttcggaacaatttatatctgctagttacttatgtgctattcctattgtccccgggcctgaattatccgatgctcgtctcgtgtacgcgaaatacgtcatgctcttgactattgtcgatgatcatttcgagagttttgcatctacagatgaatgtctcaacatcattgaattagtagaaaggtgggatgactatgcaagtgtaggttataaatctgagagggttaaagttttattttcaatgttttacaaatcaatagaggagattgcaacaattgctgaaattaaacaaggacgatctgtcaaaaatcaccttattaatttgtggcttaaagtgatgaagttgatgttgatggaacgagtagagtggtgttctggcaagacaataccaagaatagaagagtatttgtatgttagttctataacatttggttcaagattgattcctctcacaacacaatattttattggaataaaaatatccaaagatcttttagaaagtgatgaaatttatggtttatgcaattttaccggtatagtcttgaggctcctcaatgatttacaagattccaagagagaacaaaaggagggctcaataaatttagtcacattactaatgaaaagtatctctgaggaagaagctataatgaagatgaaggaaatcttggaaatgaaaagaagagagttatttaaaatggttttagttcaaaaaaagggaagccaattgcctcaattatgcaaagaaatattttggaggacatgcaaatgggctcatttcacttattcacaaactgatagatatagatttccagaggaaatggagaatcacattgatgaagtcttttacaaaccactcaatcattaa

SEQ ID NO: 3 - protein, 36 aa, Solanum habrochaites
MIVGYRSTIITLSHPKLGNGKTISSNAIFRRSCRVR

SEQ ID NO: 4 - DNA, 108 bp, Solanum habrochaites
atgatagttggctatagaagcacaatcataaccctttctcatcctaagctaggcaatgggaaaacaatttcatccaatgcaattttccggagatcatgtagagtaaga

SEQ ID NO: 5 - DNA, 777 bp, Solanum habrochaites
gctcgtggactcaacaagatttcatgctcactcagcttacaaaccgaaaaactttgttatgaggataatgataatgatcttgatgaagaacttatgcctaaacacattgctttgataatggatggtaataggagatgggcaaaggataagggtttagacgtatccgaaggtcacaaacatctctttccaaaattaaaagagatttgtgacatttcttctaaattgggaatacaagttatcactgcttttgcattctctactgaaaattggaaacgagccaagggggaggttgatttcttgatgcaaatgttcgaagaactctatgatgagttttcgaggtctggagtaagagtgtctattattggttgtaaaaccgacctcccaatgacattacaaaaatgcatagcattaacagaagagactacaaagggaaacaaaggacttcaccttgtgattgcactaaactatggtggatattatgacatattgcaagcaacaaaaagcattgttaataaagcaatgaatggtttattagatgtagaaaatatcaacaagaatttatttgatcaagaacttgaaagcaagtgtccaaatcctgatttacttataaggacaggaggtgttcaaagagttagtaactttttgttgtggcaattggcttatactgaattttacttcaccaaaacattgtttcctgattttggagaggaagatcttaaagaggcaataataaactttcaacaaaggcatagacgttttggtggacacacatattga

SEQ ID NO: 6 - protein, 258 aa, Solanum habrochaites
ARGLNKISCSLSLQTEKLCYEDNDNDLDEELMPKHIALIMDGNRRWAKDKGLDVSEGHKHLFPKLKEICDISSKLGIQVITAFAFSTENWKRAKGEVDFLMQMFEELYDEFSRSGVRVSIIGCKTDLPMTLQKCIALTEETTKGNKGLHLVIALNYGGYYDILQATKSIVNKAMNGLLDVENINKNLFDQELESKCPNPDLLIRTGGVQRVSNFLLWQLAYTEFYFTKTLFPDFGEEDLKEAIINFQQRHRRFGGHTY

SEQ ID NO: 7 - protein, 45 aa, Solanum habrochaites
MSSLVLQCWKLSSPSLILQQNTSISMGAFKGIHKLQIPNSPLTVS

SEQ ID NO: 8 - DNA, 135 bp, Solanum habrochaites
atgagttctttggttcttcaatgttggaaattatcatctccatctctgattttacaacaaaatacatcaatatccatgggtgcattcaaaggtattcataaacttcaaatcccaaattcacctctgacagtgtct